European Patent Specification EP 3 505 935 B1, published March 1, 2023. Title: Verfahren zur Diagnose einer Bornavirus-Infektion. Applicant: Euroimmun Medizinische Labordiagnostika AG. The sequence listing filed with the application follows.

SEQUENCE LISTING (7 sequences)

SEQ ID NO: 1 - protein, 382 aa, Artificial Sequence
  VSBV-N (40 kDa, His-Tag)
MNITMPPKRRLLEDPDVMDDQEPEPTSPPMPKLPGKFLQYTVGGSDPHPGIGEEKDIKHNAVALLDSSRRDMFHPVTPSLVFLCLLIPGLHAAFLHGGVPKESYLSTPISRGEQTFVKVSRFYGERTASRELTELEISSIFNHCCSLLIGVVIGSSAKIRAGAEQIKKRFKTLMASLNRPSHGETATLLQMFNPHEAIDWINGQPWVGSLVLSLLTTDFESPGKEFMDQIKLVASYAQMTTYTTIKEYLAECMDATLTIPAVAHEIREFLEISAKLKNEHAELFPFLGAIRHPDAIKLAPRSFPNLASAAFYWSKKENPTMAGYRASTIQPGATVKETQLARYRRREVSRGEDGAELSGEISDIMKMIGVTGLVLEHHHHHH

SEQ ID NO: 2 - protein, 253 aa, Artificial Sequence
  VSBV-N Peptid (30 kDa, His-GST-Tag)
MSHHHHHHHHMSPILGYWKIKGLVQPTRLLLEYLEEKYEEHLYERDEGDKWRNKKFELGLEFPNLPYYIDGDVKLTQSMAIIRYIADKHNMLGGCPKERAEISMLEGAVLDIRYGVSRIAYSKDFETLKVDFLSKLPEMLKMFEDRLCHKTYLNGDHVTHPDFMLYDALDVVLYMDPMCLDAFPKLVCFKKRIEAIPQIDKYLKSSKYIAWPLQGWQATFGGGDHPPKLEVLFQGPAMFVKVSRFYGERTASR

SEQ ID NO: 3 - protein, 210 aa, Artificial Sequence
  VSBV-P (23 kDa, His-Tag)
MASRPSSLVESLEDEESLQTPRRVRSRSPRPKRIPQDALTQPVDRLLKNIKKNPSMISDPEQRTGREQLSNDELIKQLVTELAENSMIEAEGLRGALDDISSKVDSGLESISSLQVETLQTVQKTDYADSIKTLGENIKVLDRSMKTMMETMRLMMEKIDLLYASTAIGQSNTPMLPSHPAQPRLYPTLPSAPTADEWDILPLEHHHHHH

SEQ ID NO: 4 - protein, 382 aa, Artificial Sequence
  BoDV-N (40 kDa, His-Tag)
MNITMPPKRRLVDDADAMEDQDLYEPPASLPKLPGKFLQYTVGGSDPHPGIGHEKDIRQNAVALLDQSRRDMFHTVTPSLVFLCLLIPGLHAAFVHGGVPRESYLSTPVTRGEQTVVKTAKFYGEKTTQRDLTELEISSIFSHCCSLLIGVVIGSSSKIKAGAEQIKKRFKTMMAALNRPSHGETATLLQMFNPHEAIDWINGQPWVGSFVLSLLTTDFESPGKEFMDQIKLVASYAQMTTYTTIKEYLAECMDATLTIPVVAYEIRDFLEVSAKLKEEHADLFPFLGAIRHPDAIKLAPRSFPNLASAAFYWSKKENPTMAGYRASTIQPGASVKETQLARYRRREISRGEDGAELSGEVSAIMKMIGVTGLNLEHHHHHH

SEQ ID NO: 5 - protein, 209 aa, Artificial Sequence
  BoDV-P (23 kDa, His-Tag)
MATRPSSLVDSLEDEEDPQTLRRERSGSPRPRKIPRNALTQPVDQLLKDLRKNPSMISDPDQRTGREQLSNDELIKKLVTELAENSMIEAEEVRGTLGDISARIEAGFESLSALQVETIQTAQRCDHSDSIRILGENIKILDRSMKTMMETMKLMMEKVDLLYASTAVGTSAPMLPSHPAPPRIYPQLPSAPTADEWDIIPLEHHHHHH

SEQ ID NO: 6 - protein, 15 aa, Artificial Sequence
  VSBV-N-Peptid, Aminosäuren 116-130 von A0A0H5BWD6
FVKVSRFYGERTASR

SEQ ID NO: 7 - protein, 938 aa, Artificial
  NR1 NMDAR
MSTMHLLTFALLFSCSFARAACDPKIVNIGAVLSTRKHEQMFREAVNQANKRHGSWKIQLNATSVTHKPNAIQMALSVCEDLISSQVYAILVSHPPTPNDHFTPTPVSYTAGFYRIPVLGLTTRMSIYSDKSIHLSFLRTVPPYSHQSSVWFEMMRVYNWNHIILLVSDDHEGRAAQKRLETLLEERESKAEKVLQFDPGTKNVTALLMEARELEARVIILSASEDDAATVYRAAAMLNMTGSGYVWLVGEREISGNALRYAPDGIIGLQLINGKNESAHISDAVGVVAQAVHELLEKENITDPPRGCVGNTNIWKTGPLFKRVLMSSKYADGVTGRVEFNEDGDRKFANYSIMNLQNRKLVQVGIYNGTHVIPNDRKIIWPGGETEKPRGYQMSTRLKIVTIHQEPFVYVKPTMSDGTCKEEFTVNGDPVKKVICTGPNDTSPGSPRHTVPQCCYGFCIDLLIKLARTMNFTYEVHLVADGKFGTQERVNNSNKKEWNGMMGELLSGQADMIVAPLTINNERAQYIEFSKPFKYQGLTILVKKEIPRSTLDSFMQPFQSTLWLLVGLSVHVVAVMLYLLDRFSPFGRFKVNSEEEEEDALTLSSAMWFSWGVLLNSGIGEGAPRSFSARILGMVWAGFAMIIVASYTANLAAFLVLDRPEERITGINDPRLRNPSDKFIYATVKQSSVDIYFRRQVELSTMYRHMEKHNYESAAEAIQAVRDNKLHAFIWDSAVLEFEASQKCDLVTTGELFFRSGFGIGMRKDSPWKQNVSLSILKSHENGFMEDLDKTWVRYQECDSRSNAPATLTFENMAGVFMLVAGGIVAGIFLIFIEIAYKRHKDARRKQMQLAFAAVNVWRKNLQDRKSGRAEPDPKKKATFRAITSTLASSFKRRRSSKDTSTGGGRGALQNQKDTVLPRRAIEREEGQLQLCSRHRES